European Patent Application EP 4 299 734 A1, published January 3, 2024. Title: CELL LINE FOR DISCOVERING TCR ANTIGENS AND USES THEREOF. Applicant: ETH Zurich. Application EP. The sequence listing filed with the application follows.

SEQUENCE LISTING (60 sequences)

SEQ ID NO: 1 - RNA, 20 nt, synthetic construct
  source 1..20: mol_type = other RNA
ctgcggagatcacactgacc

SEQ ID NO: 2 - DNA, 17 bp, synthetic construct
  source 1..17: mol_type = other DNA
ggttttcctggaaagtt

SEQ ID NO: 3 - DNA, 15 bp, synthetic construct
  source 1..15: mol_type = other DNA
agttctgagaaaagt

SEQ ID NO: 4 - protein, 347 aa, Homo sapiens
LNTTILTPNGNEDTTADFFLTTMPTDSLSVSTLPLPEVQCFVFNVEYMNCTWNSSSEPQPTNLTLHYWYKNSDNDKVQKCSHYLFSEEITSGCQLQKKEIHLYQTFVVQLQDPREPRRQATQMLKLQNLVIPWAPENLTLHKLSESQLELNWNNRFLNHCLEHLVQYRTDWDHSWTEQSVDYRHKFSLPSVDGQKRYTFRVRSRFNPLCGSAQHWSEWSHPIHWGSNTSKENPFLFALEAVVISVGSMGLIISLLCVYFWLERTMPRIPTLKNLEDLVTEYHGNFSAWSGVSKGLAESLQPDYSERLCLVSEIPPKGGALGEGPGASPCNQHSPYWAPPCYTLKPET

SEQ ID NO: 5 - protein, 18 aa, synthetic construct
EGRGSLLTCGDVEENPGP

SEQ ID NO: 6 - protein, 19 aa, synthetic construct
ATNFSLLKQAGDVEENPGP

SEQ ID NO: 7 - protein, 20 aa, synthetic construct
QCTNYALLKLAGDVESNPGP

SEQ ID NO: 8 - protein, 22 aa, synthetic construct
VKQTLNFDLLKLAGDVESNPGP

SEQ ID NO: 9 - protein, 20 aa, Homo sapiens
MYRMQLLSCIALSLALVTNS

SEQ ID NO: 10 - protein, 9 aa, synthetic construct
SLLMWITQC

SEQ ID NO: 11 - protein, 10 aa, synthetic construct
ELAGIGILTV

SEQ ID NO: 12 - protein, 9 aa, synthetic construct
EVDPIGHLY

SEQ ID NO: 13 - protein, 9 aa, synthetic construct
XVDPIGHLY

SEQ ID NO: 14 - protein, 9 aa, synthetic construct
EXDPIGHLY

SEQ ID NO: 15 - protein, 9 aa, synthetic construct
EVXPIGHLY

SEQ ID NO: 16 - protein, 9 aa, synthetic construct
EVDXIGHLY

SEQ ID NO: 17 - protein, 9 aa, synthetic construct
EVDPXGHLY

SEQ ID NO: 18 - protein, 9 aa, synthetic construct
EVDPIXHLY

SEQ ID NO: 19 - protein, 9 aa, synthetic construct
EVDPIGXLY

SEQ ID NO: 20 - protein, 9 aa, synthetic construct
EVDPIGHXY

SEQ ID NO: 21 - protein, 9 aa, synthetic construct
EVDPIGHLX

SEQ ID NO: 22 - DNA, 27 bp, synthetic construct
  source 1..27: mol_type = other DNA
gaagtggaccccatcggccacttgtac

SEQ ID NO: 23 - DNA, 27 bp, synthetic construct
  source 1..27: mol_type = other DNA
nnkgtggaccccatcggccacttgtac

SEQ ID NO: 24 - DNA, 27 bp, synthetic construct
  source 1..27: mol_type = other DNA
gaannkgaccccatcggccacttgtac

SEQ ID NO: 25 - DNA, 27 bp, synthetic construct
  source 1..27: mol_type = other DNA
gaagtgnnkcccatcggccacttgtac

SEQ ID NO: 26 - DNA, 27 bp, synthetic construct
  source 1..27: mol_type = other DNA
gaagtggacnnkatcggccacttgtac

SEQ ID NO: 27 - DNA, 27 bp, synthetic construct
  source 1..27: mol_type = other DNA
gaagtggaccccnnkggccacttgtac

SEQ ID NO: 28 - DNA, 27 bp, synthetic construct
  source 1..27: mol_type = other DNA
gaagtggaccccatcnnkcacttgtac

SEQ ID NO: 29 - DNA, 27 bp, synthetic construct
  source 1..27: mol_type = other DNA
gaagtggaccccatcggcnnkttgtac

SEQ ID NO: 30 - DNA, 27 bp, synthetic construct
  source 1..27: mol_type = other DNA
gaagtggaccccatcggccacnnktac

SEQ ID NO: 31 - DNA, 27 bp, synthetic construct
  source 1..27: mol_type = other DNA
gaagtggaccccatcggccacttgnnk

SEQ ID NO: 32 - protein, 9 aa, synthetic construct
EVDPIIHLY

SEQ ID NO: 33 - protein, 9 aa, synthetic construct
EVDPIGHMY

SEQ ID NO: 34 - protein, 9 aa, synthetic construct
EVDRIGHLY

SEQ ID NO: 35 - protein, 9 aa, synthetic construct
EVDPISHLY

SEQ ID NO: 36 - protein, 9 aa, synthetic construct
EVDPIGHLN

SEQ ID NO: 37 - protein, 9 aa, synthetic construct
EVTPIGHLY

SEQ ID NO: 38 - protein, 9 aa, synthetic construct
XLLMWITQC

SEQ ID NO: 39 - protein, 9 aa, synthetic construct
SXLMWITQC

SEQ ID NO: 40 - protein, 9 aa, synthetic construct
SLXMWITQC

SEQ ID NO: 41 - protein, 9 aa, synthetic construct
SLLXWITQC

SEQ ID NO: 42 - protein, 9 aa, synthetic construct
SLLMXITQC

SEQ ID NO: 43 - protein, 9 aa, synthetic construct
SLLMWXTQC

SEQ ID NO: 44 - protein, 9 aa, synthetic construct
SLLMWIXQC

SEQ ID NO: 45 - protein, 9 aa, synthetic construct
SLLMWITXC

SEQ ID NO: 46 - protein, 9 aa, synthetic construct
SLLMWITQX

SEQ ID NO: 47 - DNA, 27 bp, synthetic construct
  source 1..27: mol_type = other DNA
tcactgctgatgtggatcacacaatgc

SEQ ID NO: 48 - DNA, 27 bp, synthetic construct
  source 1..27: mol_type = other DNA
nnkctgctgatgtggatcacacaatgc

SEQ ID NO: 49 - DNA, 27 bp, synthetic construct
  source 1..27: mol_type = other DNA
tcannkctgatgtggatcacacaatgc

SEQ ID NO: 50 - DNA, 27 bp, synthetic construct
  source 1..27: mol_type = other DNA
tcactgnnkatgtggatcacacaatgc

SEQ ID NO: 51 - DNA, 27 bp, synthetic construct
  source 1..27: mol_type = other DNA
tcactgctgnnktggatcacacaatgc

SEQ ID NO: 52 - DNA, 27 bp, synthetic construct
  source 1..27: mol_type = other DNA
tcactgctgatgnnkatcacacaatgc

SEQ ID NO: 53 - DNA, 27 bp, synthetic construct
  source 1..27: mol_type = other DNA
tcactgctgatgtggnnkacacaatgc

SEQ ID NO: 54 - DNA, 27 bp, synthetic construct
  source 1..27: mol_type = other DNA
tcactgctgatgtggatcnnkcaatgc

SEQ ID NO: 55 - DNA, 27 bp, synthetic construct
  source 1..27: mol_type = other DNA
tcactgctgatgtggatcacannktgc

SEQ ID NO: 56 - DNA, 27 bp, synthetic construct
  source 1..27: mol_type = other DNA
tcactgctgatgtggatcacacaannk

SEQ ID NO: 57 - RNA, 20 nt, synthetic construct
  source 1..20: mol_type = other RNA
tgacatcaattattatacat

SEQ ID NO: 58 - RNA, 20 nt, synthetic construct
  source 1..20: mol_type = other RNA
caactacaagacccgcgccg

SEQ ID NO: 59 - RNA, 20 nt, synthetic construct
  source 1..20: mol_type = other RNA
ggggccactagggacaggat

SEQ ID NO: 60 - RNA, 20 nt, synthetic construct
  source 1..20: mol_type = other RNA
aagtcaacttcaatgtcgga